European Patent Application EP 4 678 184 A2, published January 14, 2026. Title: ENGINEERED CHIMERIC FUSION PROTEIN COMPOSITIONS AND METHODS OF USE THEREOF. Applicant: CREATE Medicines, Inc. Application EP, filed April 30, 2020. The sequence listing filed with the application follows.

SEQUENCE LISTING (50 sequences)

SEQ ID NO: 1 - protein, 116 aa, synthetic construct
  REGION 1..116: note = Description of Artificial Sequence: Synthetic polypeptide
EIQLVQSGGGLVKPGGSVRISCAASGYTFTNYGMNWVRQAPGKGLEWMGWINTHTGEPTYADSFKGRFTFSLDDSKNTAYLQINSLRAEDTAVYFCTRRGYDWYFDVWGQGTTVTV

SEQ ID NO: 2 - protein, 107 aa, synthetic construct
  REGION 1..107: note = Description of Artificial Sequence: Synthetic polypeptide
DIQMTQSPSSLSASVGDRVTITCRASQDINSYLSWFQQKPGKAPKTLIYRANRLESGVPSRFSGSGSGTDYTLTISSLQYEDFGIYYCQQYDESPWTFGGGTKLEIK

SEQ ID NO: 3 - protein, 46 aa, synthetic construct
  REGION 1..46: note = Description of Artificial Sequence: Synthetic polypeptide
LYCRRLKIQVRKAAITSYEKSDGVYTGLSTRNQETYETLKHEKPPQ

SEQ ID NO: 4 - protein, 35 aa, synthetic construct
  REGION 1..35: note = Description of Artificial Sequence: Synthetic polypeptide
YEDMRGILYAAPQLRSIRGQPGPNHEEDADSYENM

SEQ ID NO: 5 - protein, 62 aa, synthetic construct
  REGION 1..62: note = Description of Artificial Sequence: Synthetic polypeptide
KKVAKKPTNKAPHPKQEPQEINFPDDLPGSNTAAPVQETLHGCQPVTQEDGKESRISVQERQ

SEQ ID NO: 6 - protein, 21 aa, synthetic construct
  REGION 1..21: note = Description of Artificial Sequence: Synthetic peptide
IYIWAPLAGTCGVLLLSLVIT

SEQ ID NO: 7 - protein, 62 aa, synthetic construct
  REGION 1..62: note = Description of Artificial Sequence: Synthetic polypeptide
ALSNSIMYFSHFVPVFLPAKPTTTPAPRPPTPAPTIASQPLSLRPEACRPAAGGAVHTRGLD

SEQ ID NO: 8 - protein, 130 aa, synthetic construct
  REGION 1..130: note = Description of Artificial Sequence: Synthetic polypeptide
DIQMTQSPSSLSASVGDRVTITCRASQDVNTAVAWYQQKPGKAPKLLIYSASFLYSGVPSRFSGSRSGTDFTLTISSLQPEDFATYYCQQHYTTPPTFGQGTKVEIKRTGSTSGSGKPGSGEGSEVQLVE

SEQ ID NO: 9 - protein, 108 aa, synthetic construct
  REGION 1..108: note = Description of Artificial Sequence: Synthetic polypeptide
LVQPGGSLRLSCAASGFNIKDTYIHWVRQAPGKGLEWVARIYPTNGYTRYADSVKGRFTISADTSKNTAYLQMNSLRAEDTAVYYCSRWGGDGFYAMDVWGQGTLVTV

SEQ ID NO: 10 - protein, 17 aa, synthetic construct
  REGION 1..17: note = Description of Artificial Sequence: Synthetic peptide
SSGGGGSGGGGSGGGGS

SEQ ID NO: 11 - protein, 7 aa, synthetic construct
  REGION 1..7: note = Description of Artificial Sequence: Synthetic peptide
SGGGGSG

SEQ ID NO: 12 - protein, 4 aa, synthetic construct
  REGION 1..4: note = Description of Artificial Sequence: Synthetic peptide
SGGG

SEQ ID NO: 13 - protein, 4 aa, synthetic construct
  REGION 1..4: note = Description of Artificial Sequence: Synthetic peptide
GSGS

SEQ ID NO: 14 - protein, 432 aa, synthetic construct
  REGION 1..432: note = Description of Artificial Sequence: Synthetic polypeptide
MWLQSLLLLGTVACSISEIQLVQSGGGLVKPGGSVRISCAASGYTFTNYGMNWVRQAPGKGLEWMGWINTHTGEPTYADSFKGRFTFSLDDSKNTAYLQINSLRAEDTAVYFCTRRGYDWYFDVWGQGTTVTVSSGGGGSGGGGSGGGGSDIQMTQSPSSLSASVGDRVTITCRASQDINSYLSWFQQKPGKAPKTLIYRANRLESGVPSRFSGSGSGTDYTLTISSLQYEDFGIYYCQQYDESPWTFGGGTKLEIKSGGGGSGALSNSIMYFSHFVPVFLPAKPTTTPAPRPPTPAPTIASQPLSLRPEACRPAAGGAVHTRGLDIYIWAPLAGTCGVLLLSLVITLYCRRLKIQVRKAAITSYEKSDGVYTGLSTRNQETYETLKHEKPPQGSGSYEDMRGILYAAPQLRSIRGQPGPNHEEDADSYENM

SEQ ID NO: 15 - protein, 436 aa, synthetic construct
  REGION 1..436: note = Description of Artificial Sequence: Synthetic polypeptide
MWLQSLLLLGTVACSISDIQMTQSPSSLSASVGDRVTITCRASQDVNTAVAWYQQKPGKAPKLLIYSASFLYSGVPSRFSGSRSGTDFTLTISSLQPEDFATYYCQQHYTTPPTFGQGTKVEIKRTGSTSGSGKPGSGEGSEVQLVESGGGLVQPGGSLRLSCAASGFNIKDTYIHWVRQAPGKGLEWVARIYPTNGYTRYADSVKGRFTISADTSKNTAYLQMNSLRAEDTAVYYCSRWGGDGFYAMDVWGQGTLVTVSSSGGGGSGALSNSIMYFSHFVPVFLPAKPTTTPAPRPPTPAPTIASQPLSLRPEACRPAAGGAVHTRGLDIYIWAPLAGTCGVLLLSLVITLYCRRLKIQVRKAAITSYEKSDGVYTGLSTRNQETYETLKHEKPPQGSGSYEDMRGILYAAPQLRSIRGQPGPNHEEDADSYENM

SEQ ID NO: 16 - protein, 454 aa, synthetic construct
  REGION 1..454: note = Description of Artificial Sequence: Synthetic polypeptide
MWLQSLLLLGTVACSISEIQLVQSGGGLVKPGGSVRISCAASGYTFTNYGMNWVRQAPGKGLEWMGWINTHTGEPTYADSFKGRFTFSLDDSKNTAYLQINSLRAEDTAVYFCTRRGYDWYFDVWGQGTTVTVSSGGGGSGGGGSGGGGSDIQMTQSPSSLSASVGDRVTITCRASQDINSYLSWFQQKPGKAPKTLIYRANRLESGVPSRFSGSGSGTDYTLTISSLQYEDFGIYYCQQYDESPWTFGGGTKLEIKSGGGGSGALSNSIMYFSHFVPVFLPAKPTTTPAPRPPTPAPTIASQPLSLRPEACRPAAGGAVHTRGLDIYIWAPLAGTCGVLLLSLVITLYCRLKIQVRKAAITSYEKSDGVYTGLSTRNQETYETLKHEKPPQKKVAKKPTNKAPHPKQEPQEINFPDDLPGSNTAAPVQETLHGCQPVTQEDGKESRISVQERQ

SEQ ID NO: 17 - protein, 17 aa, synthetic construct
  REGION 1..17: note = Description of Artificial Sequence: Synthetic peptide
MWLQSLLLLGTVACSIS

SEQ ID NO: 18 - protein, 27 aa, synthetic construct
  REGION 1..27: note = Description of Artificial Sequence: Synthetic peptide
FWVLVVVGGVLACYSLLVTVAFIIFWV

SEQ ID NO: 19 - protein, 25 aa, synthetic construct
  REGION 1..25: note = Description of Artificial Sequence: Synthetic peptide
ILLPLIIGLILLGLLALVLIAFCII

SEQ ID NO: 20 - protein, 45 aa, synthetic construct
  REGION 1..45: note = Description of Artificial Sequence: Synthetic polypeptide
LYCRLKIQVRKAAITSYEKSDGVYTGLSTRNQETYETLKHEKPPQ

SEQ ID NO: 21 - protein, 219 aa, synthetic construct
  REGION 1..219: note = Description of Artificial Sequence: Synthetic polypeptide
QRWKSKLYSIVCGKSTPEKEGELEGTTTKPLAPNPSFSPTPGFTPTLGFSPVPSSTFTSSSTYTPGDCPNFAAPRREVAPPYQGADPILATALASDPIPNPLQKWEDSAHKPQSLDTDDPATLYAVVENVPPLRWKEFVRRLGLSDHEIDRLELQNGRCLREAQYSMLATWRRRTPRREATLELLGRVLRDMDLLGCLEDIEEALCGPAALPPAPSLLR

SEQ ID NO: 22 - protein, 171 aa, synthetic construct
  REGION 1..171: note = Description of Artificial Sequence: Synthetic polypeptide
PLCLQREAKVPHLPADKARGTQGPEQQHLLITAPSSSSSSLESSASALDRRAPTRNQPQAPGVEASGAGEARASTGSSDSSPGGHGTQVNVTCIVNVCSSSDHSSQCSSQASSTMGDTDSSPSESPKDEQVPFSKEECAFRSQLETPETLLGSTEEKPLPLGVPDAGMKPS

SEQ ID NO: 23 - protein, 211 aa, synthetic construct
  REGION 1..211: note = Description of Artificial Sequence: Synthetic polypeptide
MSNGYSTDENFRYLISCFRARVKMYIQVEPVLDYLTFLPAEVKEQIQRTVATSGNMQAVELLLSTLEKGVWHLGWTREFVEALRRTGSPLAARYMNPELTDLPSPSFENAHDEYLQLLNLLQPTLVDKLLVRDVLDKCMEEELLTIEDRNRIAAAENNGNESGVRELLKRIVQKENWFSAFLNVLRQTGNNELVQELTGSDCSESNAEIEN

SEQ ID NO: 24 - protein, 607 aa, synthetic construct
  REGION 1..607: note = Description of Artificial Sequence: Synthetic polypeptide
MWLQSLLLLGTVACSISEIQLVQSGGGLVKPGGSVRISCAASGYTFTNYGMNWVRQAPGKGLEWMGWINTHTGEPTYADSFKGRFTFSLDDSKNTAYLQINSLRAEDTAVYFCTRRGYDWYFDVWGQGTTVTVSSGGGGSGGGGSGGGGSDIQMTQSPSSLSASVGDRVTITCRASQDINSYLSWFQQKPGKAPKTLIYRANRLESGVPSRFSGSGSGTDYTLTISSLQYEDFGIYYCQQYDESPWTFGGGTKLEIKSGGGGSGALSNSIMYFSHFVPVFLPAKPTTTPAPRPPTPAPTIASQPLSLRPEACRPAAGGAVHTRGLDIYIWAPLAGTCGVLLLSLVITLYCRLKIQVRKAAITSYEKSDGVYTGLSTRNQETYETLKHEKPPQGSGSMSNGYSTDENFRYLISCFRARVKMYIQVEPVLDYLTFLPAEVKEQIQRTVATSGNMQAVELLLSTLEKGVWHLGWTREFVEALRRTGSPLAARYMNPELTDLPSPSFENAHDEYLQLLNLLQPTLVDKLLVRDVLDKCMEEELLTIEDRNRIAAAENNGNESGVRELLKRIVQKENWFSAFLNVLRQTGNNELVQELTGSDCSESNAEIEN

SEQ ID NO: 25 - protein, 615 aa, synthetic construct
  REGION 1..615: note = Description of Artificial Sequence: Synthetic polypeptide
MWLQSLLLLGTVACSISEIQLVQSGGGLVKPGGSVRISCAASGYTFTNYGMNWVRQAPGKGLEWMGWINTHTGEPTYADSFKGRFTFSLDDSKNTAYLQINSLRAEDTAVYFCTRRGYDWYFDVWGQGTTVTVSSGGGGSGGGGSGGGGSDIQMTQSPSSLSASVGDRVTITCRASQDINSYLSWFQQKPGKAPKTLIYRANRLESGVPSRFSGSGSGTDYTLTISSLQYEDFGIYYCQQYDESPWTFGGGTKLEIKSGGGGSGALSNSIMYFSHFVPVFLPAKPTTTPAPRPPTPAPTIASQPLSLRPEACRPAAGGAVHTRGLDIYIWAPLAGTCGVLLLSLVITLYCRLKIQVRKAAITSYEKSDGVYTGLSTRNQETYETLKHEKPPQGSGSQRWKSKLYSIVCGKSTPEKEGELEGTTTKPLAPNPSFSPTPGFTPTLGFSPVPSSTFTSSSTYTPGDCPNFAAPRREVAPPYQGADPILATALASDPIPNPLQKWEDSAHKPQSLDTDDPATLYAVVENVPPLRWKEFVRRLGLSDHEIDRLELQNGRCLREAQYSMLATWRRRTPRREATLELLGRVLRDMDLLGCLEDIEEALCGPAALPPAPSLLR

SEQ ID NO: 26 - protein, 567 aa, synthetic construct
  REGION 1..567: note = Description of Artificial Sequence: Synthetic polypeptide
MWLQSLLLLGTVACSISEIQLVQSGGGLVKPGGSVRISCAASGYTFTNYGMNWVRQAPGKGLEWMGWINTHTGEPTYADSFKGRFTFSLDDSKNTAYLQINSLRAEDTAVYFCTRRGYDWYFDVWGQGTTVTVSSGGGGSGGGGSGGGGSDIQMTQSPSSLSASVGDRVTITCRASQDINSYLSWFQQKPGKAPKTLIYRANRLESGVPSRFSGSGSGTDYTLTISSLQYEDFGIYYCQQYDESPWTFGGGTKLEIKSGGGGSGALSNSIMYFSHFVPVFLPAKPTTTPAPRPPTPAPTIASQPLSLRPEACRPAAGGAVHTRGLDIYIWAPLAGTCGVLLLSLVITLYCRLKIQVRKAAITSYEKSDGVYTGLSTRNQETYETLKHEKPPQGSGSPLCLQREAKVPHLPADKARGTQGPEQQHLLITAPSSSSSSLESSASALDRRAPTRNQPQAPGVEASGAGEARASTGSSDSSPGGHGTQVNVTCIVNVCSSSDHSSQCSSQASSTMGDTDSSPSESPKDEQVPFSKEECAFRSQLETPETLLGSTEEKPLPLGVPDAGMKPS

SEQ ID NO: 27 - protein, 42 aa, synthetic construct
  REGION 1..42: note = Description of Artificial Sequence: Synthetic polypeptide
RLKIQVRKAAITSYEKSDGVYTGLSTRNQETYETLKHEKPPQ

SEQ ID NO: 28 - protein, 42 aa, synthetic construct; identical to SEQ ID NO: 27
  REGION 1..42: note = Description of Artificial Sequence: Synthetic polypeptide

SEQ ID NO: 29 - protein, 24 aa, synthetic construct
  REGION 1..24: note = Description of Artificial Sequence: Synthetic peptide
IYIWAPLAGTCGVLLLSLVITLYC

SEQ ID NO: 30 - protein, 86 aa, synthetic construct
  REGION 1..86: note = Description of Artificial Sequence: Synthetic polypeptide
ALSNSIMYFSHFVPVFLPAKPTTTPAPRPPTPAPTIASQPLSLRPEACRPAAGGAVHTRGLDIYIWAPLAGTCGVLLLSLVITLYC

SEQ ID NO: 31 - protein, 83 aa, synthetic construct
  REGION 1..83: note = Description of Artificial Sequence: Synthetic polypeptide
ALSNSIMYFSHFVPVFLPAKPTTTPAPRPPTPAPTIASQPLSLRPEACRPAAGGAVHTRGLDIYIWAPLAGTCGVLLLSLVIT

SEQ ID NO: 32 - protein, 255 aa, synthetic construct
  REGION 1..255: note = Description of Artificial Sequence: Synthetic polypeptide
DIQMTQSPSSLSASVGDRVTITCRASQDVNTAVAWYQQKPGKAPKLLIYSASFLYSGVPSRFSGSRSGTDFTLTISSLQPEDFATYYCQQHYTTPPTFGQGTKVEIKRTGSTSGSGKPGSGEGSEVQLVESSGGGGSGGGGSGGGGSLVQPGGSLRLSCAASGFNIKDTYIHWVRQAPGKGLEWVARIYPTNGYTRYADSVKGRFTISADTSKNTAYLQMNSLRAEDTAVYYCSRWGGDGFYAMDVWGQGTLVTV

SEQ ID NO: 33 - protein, 240 aa, synthetic construct
  REGION 1..240: note = Description of Artificial Sequence: Synthetic polypeptide
EIQLVQSGGGLVKPGGSVRISCAASGYTFTNYGMNWVRQAPGKGLEWMGWINTHTGEPTYADSFKGRFTFSLDDSKNTAYLQINSLRAEDTAVYFCTRRGYDWYFDVWGQGTTVTVSSGGGGSGGGGSGGGGSDIQMTQSPSSLSASVGDRVTITCRASQDINSYLSWFQQKPGKAPKTLIYRANRLESGVPSRFSGSGSGTDYTLTISSLQYEDFGIYYCQQYDESPWTFGGGTKLEIK

SEQ ID NO: 34 - protein, 26 aa, synthetic construct
  REGION 1..26: note = Description of Artificial Sequence: Synthetic peptide
IYLIIGICGGGSLLMVFVALLVFYIT

SEQ ID NO: 35 - RNA, 13 nt, synthetic construct
  misc_feature 1..13: note = Description of Artificial Sequence: Synthetic oligonucleotide
  source 1..13: mol_type = other RNA
wwwtatttatttw

SEQ ID NO: 36 - protein, 44 aa, Homo sapiens
MRNKKILKEDELLSETQQAAFHQIAMEPFEINVPKPKRRNGVNF

SEQ ID NO: 37 - protein, 50 aa, Homo sapiens
MEQWDHFHNQQEDTDSCSESVKFDARSMTALLPPNPKNSPSLQEKLKSFK

SEQ ID NO: 38 - protein, 56 aa, Homo sapiens
MKVRSAGGDGDALCVTEEDLAGDDEDMPTFPCTQKGRPGPRCSRCQKNLSLHTSVR

SEQ ID NO: 39 - protein, 33 aa, synthetic construct
  REGION 1..33: note = Description of Artificial Sequence: Synthetic polypeptide
GAAPAAAPAKQEAAAPAPAAKAEAPAAAPAAKA

SEQ ID NO: 40 - protein, 20 aa, synthetic construct
  REGION 1..20: note = Description of Artificial Sequence: Synthetic peptide
  REGION 1..20: note = MISC_FEATURE - This sequence may encompass 1-4 "Gly Gly Gly Gly Ser" repeating units
  REGION 1..20: note = See specification as filed for detailed description of substitutions and preferred embodiments
GGGGSGGGGSGGGGSGGGGS

SEQ ID NO: 41 - protein, 6 aa, synthetic construct
  REGION 1..6: note = Description of Artificial Sequence: Synthetic peptide
GGGGGG

SEQ ID NO: 42 - protein, 8 aa, synthetic construct
  REGION 1..8: note = Description of Artificial Sequence: Synthetic peptide
GGGGGGGG

SEQ ID NO: 43 - protein, 20 aa, synthetic construct
  REGION 1..20: note = Description of Artificial Sequence: Synthetic peptide
  REGION 1..20: note = MISC_FEATURE - This sequence may encompass 1-4 "Glu Ala Ala Ala Lys" repeating units
  REGION 1..20: note = See specification as filed for detailed description of substitutions and preferred embodiments
EAAAKEAAAKEAAAKEAAAK

SEQ ID NO: 44 - protein, 4 aa, synthetic construct
  REGION 1..4: note = Description of Artificial Sequence: Synthetic peptide
GGGS

SEQ ID NO: 45 - protein, 5 aa, synthetic construct
  REGION 1..5: note = Description of Artificial Sequence: Synthetic peptide
GGGGS

SEQ ID NO: 46 - protein, 5 aa, synthetic construct
  REGION 1..5: note = Description of Artificial Sequence: Synthetic peptide
EAAAK

SEQ ID NO: 47 - protein, 4 aa, synthetic construct
  REGION 1..4: note = Description of Artificial Sequence: Synthetic peptide
SGGS

SEQ ID NO: 48 - protein, 16 aa, synthetic construct
  REGION 1..16: note = Description of Artificial Sequence: Synthetic peptide
SGSETPGTSESATPES

SEQ ID NO: 49 - protein, 21 aa, synthetic construct
  REGION 1..21: note = Description of Artificial Sequence: Synthetic peptide
  REGION 1..21: note = MISC_FEATURE - This sequence may encompass 1, 3, or 7 "Gly Gly Ser" repeating units
GGSGGSGGSGGSGGSGGSGGS

SEQ ID NO: 50 - protein, 12 aa, unidentified
  REGION 1..12: note = Description of Unknown: hinge region sequence
ESKYGPPCPPCP